European Patent Application EP 4 201 959 A1, published June 28, 2023. Title: PROTEIN, POLYNUCLEOTIDE, VECTOR, HOST CELL, COMPOSITION, METHOD FOR TREATING AN ILLNESS, IN-VITRO METHOD FOR PREDICTING MULTIPLE SCLEROSIS, AND USE OF A PROTEIN OR COMPOSITION. Applicant: Fundacao Oswaldo Cruz. The sequence listing filed with the application follows.

SEQUENCE LISTING (15 sequences)

SEQ ID NO: 1 - DNA, 711 bp, Artificial Sequence
  scFv anti-VLA-4
gacgtggtgatgacccagagccccctgagcctgcccgtgacccccggcgagcccgccagcatcagctgcaggagcagccagagcctggccaagagctacagcaacacctacctgagctggtacctgcagaagcccggccagagcccccagctgctgatctacggcatcggcaacggcggcagcggcgtgcccgccaggttcagcggcagcggcagcggcaccgacttcaccctgctgatcagcagggtggaggccgaggacgtgggcgtgtactactgcctgcagggcacccaccagccctacaccttcggccagggcaccaaggtggagatcggcggcggcggcagccaggtgcagctggtgcagagcggcgccgaggtgaagaagcccggcgccagcgtgaaggtgagctgcaagggcagcggctacaccttcaccagctactggatgcactgggtgaggcaggcccccggccagaggctggagtggatcggcgagatcggccccagcgagagcaacaccaactacaaccagaagttcaagggcagggtgaccctgaccgtggacatcagcgccagcaccgcctacatggagctgagcagcctgaggagcgaggacaccgccgtgtactactgcgccaggggcggctacgccggctgggactacgccatcgactactggggccagggcaccctggtgaccgtgagcagc

SEQ ID NO: 2 - DNA, 711 bp, Artificial Sequence
  scFv anti-VLA-4
gacgttgtaatgactcaatcgccactttctttacctgtaactcccggtgaacctgcgtctatttcgtgtcgcagtagtcagtctctggccaagtcttattccaatacttacctgtcctggtatcttcaaaagcctggacagtcaccacaacttttaatatatggcattgggaatggcgggagtggagtgcctgctcgtttcagcggctctggtagcggaacagacttcacattactgattagtcgtgtcgaagctgaagacgttggagtgtactactgcttgcaagggacccatcagccttacacgtttggccaaggcactaaagtggagataggcggcggcggcagtcaggttcagttagtccaaagtggggccgaggttaagaagcccggcgcttctgtcaaagtctcgtgtaagggcagtggctacacgttcacatcatactggatgcactgggtacggcaagctcctggtcagagactggagtggatcggcgagattggaccctccgagagcaatacgaactataaccaaaaattcaaaggacgcgtcacactgacggtcgacatatctgcttcgacggcatacatggaattaagttctcttagaagtgaagacacggcagtatattactgcgctcgtggaggatatgctggttgggactacgcgattgactactggggccaaggtactcttgtcacggtcagtagc

SEQ ID NO: 3 - protein, 237 aa, Artificial Sequence
  scFv anti-VLA-4
DVVMTQSPLSLPVTPGEPASISCRSSQSLAKSYSNTYLSWYLQKPGQSPQLLIYGIGNGGSGVPARFSGSGSGTDFTLLISRVEAEDVGVYYCLQGTHQPYTFGQGTKVEIGGGGSQVQLVQSGAEVKKPGASVKVSCKGSGYTFTSYWMHWVRQAPGQRLEWIGEIGPSESNTNYNQKFKGRVTLTVDISASTAYMELSSLRSEDTAVYYCARGGYAGWDYAIDYWGQGTLVTVSS

SEQ ID NO: 4 - protein, 243 aa, Artificial Sequence
  scFv anti-VLA-4
DVVMTQSPLSLPVTPGEPASISCRSSQSLAKSYSNTYLSWYLQKPGQSPQLLIYGIGNGGSGVPARFSGSGSGTDFTLLISRVEAEDVGVYYCLQGTHQPYTFGQGTKVEIGGGGSQVQLVQSGAEVKKPGASVKVSCKGSGYTFTSYWMHWVRQAPGQRLEWIGEIGPSESNTNYNQKFKGRVTLTVDISASTAYMELSSLRSEDTAVYYCARGGYAGWDYAIDYWGQGTLVTVSSHHHHHH

SEQ ID NO: 5 - protein, 111 aa, Artificial Sequence
  scFv anti-VLA-4
DVVMTQSPLSLPVTPGEPASISCRSSQSLAKSYSNTYLSWYLQKPGQSPQLLIYGIGNGGSGVPARFSGSGSGTDFTLLISRVEAEDVGVYYCLQGTHQPYTFGQGTKVEI

SEQ ID NO: 6 - protein, 121 aa, Artificial Sequence
  scFv anti-VLA-4
QVQLVQSGAEVKKPGASVKVSCKGSGYTFTSYWMHWVRQAPGQRLEWIGEIGPSESNTNYNQKFKGRVTLTVDISASTAYMELSSLRSEDTAVYYCARGGYAGWDYAIDYWGQGTLVTVSS

SEQ ID NO: 7 - protein, 19 aa, Artificial Sequence
  scFv anti-VLA-4
SCRSSQSLAKSYSNTYLSW

SEQ ID NO: 8 - protein, 13 aa, Artificial Sequence
  scFv anti-VLA-4
LIYGIGNGGSGVP

SEQ ID NO: 9 - protein, 10 aa, Artificial Sequence
  scFv anti-VLA-4
LQGTHQPYTF

SEQ ID NO: 10 - protein, 11 aa, Artificial Sequence
  scFv anti-VLA-4
SGYTFTSYWMH

SEQ ID NO: 11 - protein, 19 aa, Artificial Sequence
  scFv anti-VLA-4
EIGPSESNTNYNQKFKGRV

SEQ ID NO: 12 - protein, 14 aa, Artificial Sequence
  scFv anti-VLA-4
GGYAGWDYAIDYWG

SEQ ID NO: 13 - protein, 5 aa, Artificial Sequence
  scFv anti-VLA-4
GGGGS

SEQ ID NO: 14 - protein, 10 aa, Artificial Sequence
  scFv anti-VLA-4
GGGGSGGGGS

SEQ ID NO: 15 - protein, 15 aa, Artificial Sequence
  scFv anti-VLA-4
GGGGSGGGGSGGGGS